European Patent Application EP 4 242 224 A1, published September 13, 2023. Title: Antibodies specific for coronavirus spike protein and uses thereof. Applicant: GREEN CROSS CORPORATION Mogam Institute for Biomedical Research. The sequence listing filed with the application follows.

SEQUENCE LISTING (169 sequences)

SEQ ID NO: 1 - DNA, 753 bp, Unknown
  SARS Corona virus 2 spike protein RBD domain
atgtttgtgtttctggttctgctgcccctggtgtcctctagagtgcagcctacagagtccatcgtgcggttccccaacatcaccaatctgtgccctttcggcgaggtgttcaacgccacaagatttgccagcgtgtacgcctggaaccggaagagaatcagcaactgcgtggccgactacagcgtgctgtacaatagcgccagcttcagcaccttcaagtgctacggcgtgtcccctaccaagctgaacgacctgtgcttcaccaatgtgtacgccgacagcttcgtgatcagaggcgacgaagttcggcagatcgctcctggacagacaggcaagatcgccgattacaactacaagctgcccgacgacttcaccggctgcgtgatcgcctggaatagcaacaacctggacagcaaagtcggcggcaactacaactacctgtaccggctgttccggaagtccaacctgaagcctttcgagcgggacatcagcaccgagatctatcaggccggcagcaccccttgtaatggcgtggaaggcttcaactgctacttcccactgcagtcctacggcttccagcctacaaacggcgtgggctaccagccttatagagtggtggtgctgagcttcgaactgctgcatgcccctgctaccgtgtgcggccctaagaagtctaccaacctggtcaagaacaaatgcgtgaacttcggcggcctggtgcctagaggatctcaccaccatcaccatcactaa

SEQ ID NO: 2 - protein, 250 aa, Unknown
  SARS Corona virus 2 spike protein RBD domain
MFVFLVLLPLVSSRVQPTESIVRFPNITNLCPFGEVFNATRFASVYAWNRKRISNCVADYSVLYNSASFSTFKCYGVSPTKLNDLCFTNVYADSFVIRGDEVRQIAPGQTGKIADYNYKLPDDFTGCVIAWNSNNLDSKVGGNYNYLYRLFRKSNLKPFERDISTEIYQAGSTPCNGVEGFNCYFPLQSYGFQPTNGVGYQPYRVVVLSFELLHAPATVCGPKKSTNLVKNKCVNFGGLVPRGSHHHHHH

SEQ ID NO: 3 - DNA, 1620 bp, Unknown
  SARS Corona virus 2 spike protein RBD-SD1-Fc
atgcggcctacttgggcctggtggctgttcctggtgctgctgctagctctgtgggcacccgctagagggcgggtgcagcctacagagagcatcgtgcgatttccaaacattaccaacctctgccccttcggcgaggtgtttaacgccacaagatttgcctccgtttacgcctggaatagaaagagaatcagcaattgtgtggccgactactccgtgctgtataacagcgcctctttcagcaccttcaagtgctacggcgtttccccaacaaagctgaatgacctgtgcttcaccaacgtgtacgccgactccttcgtaattagaggcgatgaggtgcggcagatcgcaccaggccagaccggtaagatcgctgactacaactataagctgcctgatgattttacaggctgcgtgatcgcctggaactctaacaacctggatagcaaggtgggcggcaactacaactacctgtaccggctgtttcgcaagtctaacctgaaacctttcgagagagacatctccacagagatctaccaggccggttctacaccttgtaacggggtggaaggcttcaactgttacttccctctgcaaagctacggcttccagcctaccaatggagtcggctaccagccataccgggtggtcgtgctgtccttcgagttactccacgcccccgccaccgtctgcggtcctaagaagtccaccaatctggttaagaacaaatgcgtgaacttcaacttcaacggcctgaccgggaccggcgtgctgaccgaaagcaacaaaaagttcctccccttccagcagttcggccgtgatatcgctgacaccacagatgccgtcagagatccacagaccctggaaatcctggatattacaccctgctccggatccctggaggtgctgttccagggcccaactcacacatccccaccgagcccagcacctgaactcctggggggaccgtcagtcttcctcttccccccaaaacccaaggacaccctcatgatctcccggacccctgaggtcacatgcgtggtggtggacgtgagccacgaagaccctgaggtcaagttcaactggtacgtggacggcgtggaggtgcataatgccaagacaaagccgcgggaggagcagtacaacagcacgtaccgtgtggtcagcgtcctcaccgtcctgcaccaggactggctgaatggcaaggagtacaagtgcaaggtctccaacaaagccctcccagcccccatcgagaaaaccatctccaaagccaaagggcagccccgagaaccacaggtgtacaccaaacccccatcccgggatgagctgaccaagaaccaggtcagcctgtcctgcctggtcaaaggcttctatcccagcgacatcgccgtggagtgggagagcaatgggcagccggagaacaactacaagaccacggtccccgtgctggactccgacggctccttcaggctcgccagctatctcaccgtggacaagagcaggtggcagcaggggaacgtcttctcatgctccgtgatgcatgaggctctgcacaaccactacacgcagaagagcctctccctgtctccgggtaaacatcaccatcatcaccaccatcactag

SEQ ID NO: 4 - protein, 250 aa, Unknown; identical to SEQ ID NO: 2
  SARS Corona virus 2 spike protein RBD-SD1-Fc

SEQ ID NO: 5 - protein, 124 aa, Artificial Sequence
  heavy chain variable region of clone 1
EVQLVQSGAEVQKPGSSVKVSCKASGGTFSSYPISWVRQAPGQGLEWMGKIIPILGIPNYAQRFQGRVTITADKSTGTAYLDLSSLSSEDTAVYYCARAGGYSGYGAHYYMDVWGKGTLVTVSS

SEQ ID NO: 6 - protein, 122 aa, Artificial Sequence
  heavy chain variable region of clone 2
EVQLVESGGGLIQPGGSLRLSCAASGFTFSNFAMSWVRQAPGKGLEWVSGISGSGGSTSYADSVKGRFTISRDNSKNTLYLQMNSLRAEDTAVFYCAKDLYGGPGSSTFDYWGQGTLVTVSS

SEQ ID NO: 7 - protein, 122 aa, Artificial Sequence
  heavy chain variable region of clone 3
QVQLVQSGGGLIQPGGSLRLSCAASGFTFSNFAMSWVRQAPGKGLEWVSGISGSGGSTSYADSVKGRFTISRDNSKNTLYLQMNSLRAEDTAVFYCAKDLYGGPGSSTFDYWGQGTLVTVSS

SEQ ID NO: 8 - protein, 122 aa, Artificial Sequence
  heavy chain variable region of clone 4
EDQLVESGGGLIQPGGSLRLSCAASGFTFSNFAMSWVRQAPGKGLEWVSGISGSGGSTSYADSVKGRFTISRDNSKNTLYLQMNSLRVEDTAVFYCAKDLYGGPGSSTFDYWGQGTLVTVSS

SEQ ID NO: 9 - protein, 122 aa, Artificial Sequence
  heavy chain variable region of clone 5
EDQLVESGGGLIQPGGSLRLSCAASGFTFSNFAMSWVRQAPGKGLEWVSGISGSGGSTSYADSVKGRFTISRDNSKNTLYLQMNSLRAEDTAVFYCAKDLYGGPGSSTFDYWGQGTLVTVSS

SEQ ID NO: 10 - protein, 123 aa, Artificial Sequence
  heavy chain variable region of clone 6
QLQLQESGGGWVQPGRSLRLTCATSGFTFDDYAMHWVRQAPGKGLEWVSGITWNSDSIGYADSVKGRFTISRDDAKNSLYLQMDNLRPEDTALYYCVKDSAYRILPYWYFDLWGRGTTVTVSS

SEQ ID NO: 11 - protein, 122 aa, Artificial Sequence
  heavy chain variable region of clone 7
EVQLVESGGDLVQPGGSLRISCAASGFAVSNNYMSWVRQAPGKGLEWVSVIHTDGSTYYADSVKGRFTISRDNSKNTLYLQMNSLRAEDTAVYYCAREGFGELLGSDAFDIWGQGTMVTVSS

SEQ ID NO: 12 - protein, 122 aa, Artificial Sequence
  heavy chain variable region of clone 8
QVQLVQSGGGLVQPGGSLRLSCVASGFTFRTFEMNWVRQAPGKGLEWVSYISPSGSSIYNADSVKGRFTISRDNARNSLYLQMNSLRAEDTAVYYCAREGGSYYGGSAFDIWGQGTMVTVSS

SEQ ID NO: 13 - protein, 122 aa, Artificial Sequence
  heavy chain variable region of clone 9
EVQLVESGGGVVQPGRSLRLSCVASGFTFRTFEMNWVRQAPGKGLEWVSYISPSGSSIYNADSVKGRFTISRDNARNSLYLQMNSLRAEDTAVYYCAREGGSYYGGSAFDIWGQGTTVTVSS

SEQ ID NO: 14 - protein, 122 aa, Artificial Sequence
  heavy chain variable region of clone 10
EVQLVQSGGGSVQPGGSLRLSCAASGFTFRTFEMNWVRQAPGKGLEWVSYISPSGSSIYNADSVKGRFTISRDNARNSLYLQMNSLRAEDTAVYYCAREGGSYYGGSAFDIWGQGTMVTVSS

SEQ ID NO: 15 - protein, 129 aa, Artificial Sequence
  heavy chain variable region of clone 11
EVQLVESGGGLVQPGGSLRLSCAASGFTFSTYWMSWVRQAPGKGLEWVANIKQEGSEKYYVDSVKGRFTISRDNAKNSLYLQMNSLRAEDTAVYYCAREGGYYYGSGSYYKPKVVFDHWGQGTLVTVSS

SEQ ID NO: 16 - protein, 129 aa, Artificial Sequence
  heavy chain variable region of clone 12
EVQLVESGGGLVQPGGSLRLSCAASGFTFSTYAMSWVRQAPGKGLEWVSAISGNGGSTSYAASVQGRFTISRDNSKNTLYLQMNSLRAEDTAVYYCAREGGYYYGSGSYYKPKVVFDYWGQGTLVTVSS

SEQ ID NO: 17 - protein, 129 aa, Artificial Sequence
  heavy chain variable region of clone 13
QVQLVESGGGVVQPGRSLRLSCAASGFTFRGYAMHWVRQAPGKGLEWVAVISEDGSDEYYADSVKGRFTISRDNSKNTLYLQMNSLRAEDTAVYYCAREGGYYYGSGSYYKPKVVFDYWGQGTLVTVSS

SEQ ID NO: 18 - protein, 129 aa, Artificial Sequence
  heavy chain variable region of clone 14
EVQLVESGGGLVQPGGSLRLSCAASGFTFSTYWMSWVRQAPGKGLEWVANIKQEGSEKYYVDSVKGRFTISRDNAKNSLYLQMNSLRAEDTAVYYCAREGGYYYGSGSYYKPKVVFDYWGQGTLVTVSS

SEQ ID NO: 19 - protein, 129 aa, Artificial Sequence
  heavy chain variable region of clone 15
QVQLVESGGTLVQPGGSLRLSCAASGFTFSGYAMNWVRQAPGKGLEWVSSVSGRGDTTHYADSVKGRFTISRDNRENKLYLQMHSLRAEDTAVYYCAREGGYYYGSGSYYKPKVVFDYWGQGTLVTVSS

SEQ ID NO: 20 - protein, 129 aa, Artificial Sequence
  heavy chain variable region of clone 16
EVQLVESGGGLVQPGGSLRLSCAASGFTFRTYAMSWVRQAPGKGLEWVSAISSSDDTTYYADSVKGRFTISRDNSKNTLYLQMNSLRAEDTAVYYCAREGGYYYGSGSYYKPKVVFDYWGQGTLVTVSS

SEQ ID NO: 21 - protein, 129 aa, Artificial Sequence
  heavy chain variable region of clone 17
EVQLVESGGGLVQPGGSLRLSCAASGFSSSYYWMSWVRQAPGKGLEWVANIKQEGSEKYYVDSVKGRFTISRDNAKNSLYLQMNSLRAEDTAVYYCAREGGYYYGSGSYYKPKVVFDYWGQGTLVTVSS

SEQ ID NO: 22 - protein, 129 aa, Artificial Sequence
  heavy chain variable region of clone 18
EVQLVQSGGGLVQPGGSLRLSCAASGFTFRTYAMSWVRQAPGKGLEWVSAISSSDDTTYYADSVKGRFTISRDNSKNTLYLQMNSLRAEDTAVYYCAREGGYYYGSGSYYKPKVVFDYWGQGTLVTVSS

SEQ ID NO: 23 - protein, 129 aa, Artificial Sequence
  heavy chain variable region of clone 19
EVQLLESGGGLVQPGGSLRLSCAASGFTFSTYWMSWVRQAPGKGLEWVANIKQEGSEKYYVDSVKGRFTISRDNAKNSLYLQMNSLRAEDTAVYYCAREGGYYYGSGSYYKPKVVFDYWGQGTLVTVSS

SEQ ID NO: 24 - protein, 129 aa, Artificial Sequence
  heavy chain variable region of clone 20
EVQLVESGGGLVQPGGSLRLSCAASGFTFRTYAMSWVRQAPGKGLEWVSAISSSDDTTYYADSVKGRFTISRDNAKNSLYLQMNSLRAEDTAVYYCAREGGYYYGSGSYYKPKVVFDYWGQGTTVTVSS

SEQ ID NO: 25 - protein, 129 aa, Artificial Sequence
  heavy chain variable region of clone 21
QVQLLESGGGLVQPGGSLRLSCAASGFTFSTYWMSWVRQAPGKGLEWVANIKQEGSEKYYVDSVKGRFTISRDNAKNSLYLQMNSLRAEDTAVYYCAREGGYYYGSGSYYKPKVVFDYWGQGTLVTVSS

SEQ ID NO: 26 - protein, 129 aa, Artificial Sequence
  heavy chain variable region of clone 22
EVQLVESGGGLAQSGGSLRLSCEASGFTFSTYWMSWVRQAPGKGLEWVANIKQEGSEKYYVDSVKGRFTISRDNAKNSLYLQMNSLRAEDTAVYYCAREGGYYYGSGSYYKPKVVFDYWGQGTLVTVSS

SEQ ID NO: 27 - protein, 129 aa, Artificial Sequence
  heavy chain variable region of clone 23
QVQLVESGGGLVQPGGSLRLSCAASGFTFSTYWMSWVRQAPGKGLEWVANIKQEGSEKYYVDSVKGRFTISRDNAKNSLYLQMNSLRAEDTAVYYCAREGGYYYGSGSYYKPKVVFDYWGQGTLVTVSS

SEQ ID NO: 28 - protein, 129 aa, Artificial Sequence
  heavy chain variable region of clone 24
EVQLVESGGAMVQPGGSLRLSCAASGFTFSTYWMSWVRQAPGKGLEWVANIKQEGSEKYYVDSVKGRFTISRDNAKNSLYLQMNSLRAEDTAVYYCAREGGYYYGSGSYYKPKVVFDYWGQGTLVTVSS

SEQ ID NO: 29 - protein, 129 aa, Artificial Sequence
  heavy chain variable region of clone 25
EVQLVESGGGLVQPGGSLRLSCAASGFTFSTYWMSWVRQAPGKGLEWVANIKQEGSEKYYVDSVKGRFTISKDNAKNSLYLQMNSLRAEDTAVYYCAREGGYYYGSGSYYKPKVVFDYWGQGTLVTVSS

SEQ ID NO: 30 - protein, 129 aa, Artificial Sequence; identical to SEQ ID NO: 18
  heavy chain variable region of clone 26

SEQ ID NO: 31 - protein, 129 aa, Artificial Sequence; identical to SEQ ID NO: 18
  heavy chain variable region of clone 27

SEQ ID NO: 32 - protein, 129 aa, Artificial Sequence
  heavy chain variable region of clone 28
QVQLVQSGGGLVQPGGSLRLSCAASGFTFSTYWMSWVRQAPGKGLEWVANIKQEGSEKYYVDSVKGRFTISRDNAKNSLYLQMNSLRAEDTAVYYCAREGGYYYGSGSYYKPKVVFDYWGQGTLVTVSS

SEQ ID NO: 33 - protein, 129 aa, Artificial Sequence; identical to SEQ ID NO: 27
  heavy chain variable region of clone 29

SEQ ID NO: 34 - protein, 129 aa, Artificial Sequence
  heavy chain variable region of clone 30
EVQLVETGGGLVQPGGSLRLSCAASGFTFSTYWMSWVRQAPGKGLEWVANIKQEGSEKYYVDSVKGRFTISRDNAKNSLYLQMNSLRAEDTAVYYCAREGGYYYGSGSYYKPKVVFDYWGQGTLVTVSS

SEQ ID NO: 35 - protein, 129 aa, Artificial Sequence; identical to SEQ ID NO: 18
  heavy chain variable region of clone 31

SEQ ID NO: 36 - protein, 129 aa, Artificial Sequence
  heavy chain variable region of clone 32
QVQLVQSGGGVVQPGGSLRLSCAASGFTFSGYGMNWVRQAPGKGLEWVADIEKDGGERNYADSVKGRFTISRDNAKNSLYLQMNSLRAEDTAVYYCAREGGYYYGSGSYYKPKVVFDYWGQGTLVTVSS

SEQ ID NO: 37 - protein, 133 aa, Artificial Sequence
  heavy chain variable region of clone 33
EVQLVESGGGLIQPGGSLRLSCAASGFTFSSFWMSWVRQAPGKGLEWVANIKQDGSEKYSVDSVKGRFTISRDNAKNSLYLQMNSLRAEDTAVYYCARHGIYCSGDNCYYFAPTLSSHAFDIWGQGTMVTVSS

SEQ ID NO: 38 - protein, 125 aa, Artificial Sequence
  heavy chain variable region of clone 34
QVQLVQSGGGLVQPGRSLRLSCAASGFTFDDYAMHWVRQAPGKGLEWVSGSSWNSGTIGYADSVKGRFTISRDNAKNSLYLQMNSLRAEDTALYYCAIIPGDGYNYPGASDFDYWGQGTLVTVSS

SEQ ID NO: 39 - protein, 125 aa, Artificial Sequence
  heavy chain variable region of clone 35
EVQLLESGGGLVQPGRSLKLSCAASGFTFDDYAMHWVRQAPGKGLEWVSGSSWNSGTIGYADSVKGRFTISRDNAKNSLYLQMNSLRAEDTALYYCAIIPGDGYNYPGASDFDYWGQGTLVTVSS

SEQ ID NO: 40 - protein, 125 aa, Artificial Sequence
  heavy chain variable region of clone 36
QVTLKESGGGLVQPGRSLRLSCAASGFTFDDYAMHWVRQAPGKGLEWVSGSSWNSGTIGYADSVKGRFTISRDNAKNSLYLQMNSLRAEDTALYYCAIIPGDGYNYPGASDFDYWGQGTLVTVSS

SEQ ID NO: 41 - protein, 125 aa, Artificial Sequence
  heavy chain variable region of clone 37
QVQLVESGGGLVQPGGSLRLSCAASGFTFDDYAMHWVRQAPGKGLEWVSGSSWNSGTIGYADSVKGRFTISRDNAKNSLYLQMNSLRAEDTALYYCAIIPGDGYNYPGASDFDYWGQGTTVTVSS

SEQ ID NO: 42 - protein, 120 aa, Artificial Sequence
  heavy chain variable region of clone 38
QVQLVQSGAEVKKPGASVRVSCKASGYTFSSYYTHWVRQAPGQGLEWMGIINPSGGSTIYAQKFQGRVTMTRDTSTSTVYMELSSLRSEDTAVYYCARLPRDGVHASDIWGQGTTVTVSS

SEQ ID NO: 43 - protein, 122 aa, Artificial Sequence
  heavy chain variable region of clone 39
EVQLVESGGGLVQPGGSLRLSCAASGFTFSTYYMGWVRQAPGKGLEWVSLISGSGGSTYYDDSVKGRFTISRDNSKNTLYLQMNSLRAEDTAVYYCAKPPYSFDSMSESDYWGQGTLVTVSS

SEQ ID NO: 44 - protein, 127 aa, Artificial Sequence
  heavy chain variable region of clone 40
QVQLQDSGPGLVKPSETLSLTCTVSGGSISSYDWSWIRQPPGKGLEWIGDIYNSGSTKYNPSLKSRVTISVDTSKNQLSLKLSSVTAADTAVYYCARRGLGNYDILTGYFENAFDIWGQGTTVTVSS

SEQ ID NO: 45 - protein, 127 aa, Artificial Sequence
  heavy chain variable region of clone 41
ETQLVESGGGLVQPGGSLRLSCAASGFTFSSYSMNWVRQAPGKGLEWVSYISSSTSTIYYADSVKGRFTISRDNAKNSLYLQMNSLRAEDTAVYYCARTRLTQLAMIGRGGNAFDIWGQGTMVTVSS

SEQ ID NO: 46 - protein, 112 aa, Artificial Sequence
  light chain variable region of clone 1
QSVLTQPPSVSGAPGQRVTISCTGSSSNIGAGYDVHWYQQLPGTAPKLLIYGNSNRPSGVPDRFSGSKSGTSASLAITGLQAEDEADYYCQSYDSSLSGSVFGGGTKLTVLG

SEQ ID NO: 47 - protein, 108 aa, Artificial Sequence
  light chain variable region of clone 2
DIVMTQSPSSLSASVGDRVTITCQASQDISNYLNWYQQKPGKAPKLLIYDASNLETGVPSRFSGSGSGTDFTFTISSLQPEDIATYYCQQYDNLPLTFGPGTKVDIKR

SEQ ID NO: 48 - protein, 108 aa, Artificial Sequence
  light chain variable region of clone 3
AIWMTQSPSSLSASVGDRVTITCQASQDISNYLNWYQQKPGKAPKLLIYDASNLETGVPSRFSGNGSGTDFTLTISSLQPEDFAIYYCQQSYSTPLTFGGGTKVEIKR

SEQ ID NO: 49 - protein, 108 aa, Artificial Sequence
  light chain variable region of clone 4
DIVMTQTPSSLSASVGDRVTITCQASQDISIYLNWYQQKPGKAPKLLIYDASILETGVPSRFSGSGSGTDFTLTISSLQPEDFATYYCQQYFSYPITFGGGTKVEIKR

SEQ ID NO: 50 - protein, 107 aa, Artificial Sequence
  light chain variable region of clone 5
DIQMTQSPSSLSASVGDRVTITCQASEDITDYLNWYQQKPGKAPKLLIYDASILETGVPSRFSGSGSGTDFTLTISSLQPEDVATYYCQQYDGLPLFGPGTKVDIKR

SEQ ID NO: 51 - protein, 108 aa, Artificial Sequence
  light chain variable region of clone 6
DIQMTQSPSSLSASVGDRVTITCRASQSISNYLNWYQQIPGKAPKLLMYAATRLHSGVPSRFSGSGSGTDFTLTIYSLQPEDFATYYCQQSFGSPYTFGQGTKLEIKR

SEQ ID NO: 52 - protein, 108 aa, Artificial Sequence
  light chain variable region of clone 7
AIQMTQSPSSLSASVGDRVTITCRASQSISSYLNWYQQKPGKAPKLLIYAASSLQSGVPSRFSGSGSGTDFTLTISSLQPEDFATYYCQQSYSTPHTFGPGTKVDIKR

SEQ ID NO: 53 - protein, 111 aa, Artificial Sequence
  light chain variable region of clone 8
SYELTQPSSASGTPGQRVTISCSGSSSNIGSNTVNWYQQLPGTAPKLLIYSNNQRPSGVPDRFSGSKSGTSASLAISGLQSEDEADYYCAAWDDSLNGWVFGGGTKLTVLG

SEQ ID NO: 54 - protein, 111 aa, Artificial Sequence
  light chain variable region of clone 9
SYELTQPPSASGTPGQRVTISCSGSSSNIERNIVNWYQQVPGTAPKLLIYTNSHRPSGVPDRFSGSKSGSAASLAISGLQSEDEADYYCAAWDDTLNGWVFGGGTKLTVLG

SEQ ID NO: 55 - protein, 112 aa, Artificial Sequence
  light chain variable region of clone 10
QSVPTQPPSASGTPGQRVTISCSGSSSNIGSNTVNWYQQLPGTAPKLLIYSNNQRPSGVPDRFSGSKSGTSASLAISGLQSEDEADYYCAAWDDSLNGRWVFGGGTKLTVLG

SEQ ID NO: 56 - protein, 111 aa, Artificial Sequence
  light chain variable region of clone 11
QSALTQPRSVSGSPGQSVTISCTGTSSDVGGYNYVSWYQQHPGKAPKLMIYDVSKRPSGVPDRFSGSKSGNTASLTISGLQAEDEADYYCCSYAGSYTWVFGGGTKLTVLG

SEQ ID NO: 57 - protein, 112 aa, Artificial Sequence
  light chain variable region of clone 12
QSVLTQPPSVSGAPGQRVTISCTGSSSNIGAGYDVHWYQQLPGTAPKLLIYGNSNRPSGVPDRFSGSKSGTSASLAITGLQAEDEADYYCQSYDSSLSGYVFGTGTKVTVLG

SEQ ID NO: 58 - protein, 112 aa, Artificial Sequence
  light chain variable region of clone 13
QSVLTQPPSVSGAPGQRVTISCTGSSSNIGAGYDVHWYQQLPGTAPKLLIYGNSNRPSGVPDRFSGSKSGTSASLAITGLQAEDEADYYCQSYDSSLSGYVFGTGTELTVLG

SEQ ID NO: 59 - protein, 112 aa, Artificial Sequence
  light chain variable region of clone 14
SYELTQPPSVSGAPGQRVTISCTGSSSNIGAGYDVHWYQQLPGTAPKLLIYGNSNRPSGVPDRFSGSKSGTSASLAITGLQAEDEADYYCQSYDSSLSGYVFGTGTKVTVLG

SEQ ID NO: 60 - protein, 112 aa, Artificial Sequence
  light chain variable region of clone 15
QAGLTQPPSVSGAPGQRVTMSCTGTTSNIGAGYDVHWYQQLPGTAPKLLIYGNSNRPSGVPDRFSGSKSGTSASLAISGLQSEDEADYYCAAWDDSLNGYVFGTGTKVTVLG

SEQ ID NO: 61 - protein, 112 aa, Artificial Sequence
  light chain variable region of clone 16
SYELTQPLSVSGAPGQRVTISCTGSSSNIGAGYDVHWYQQLPGTAPKLLIYGNSNRPSGVPDRFSGSKSGTSASLAITGLQAEDEADYYCQSYDSSLSGWVFGGGTKLTVLG

SEQ ID NO: 62 - protein, 112 aa, Artificial Sequence
  light chain variable region of clone 17
QSVLTQPPSVSGAPGQRVTISCTGSSSNIGAGYDVHWYQQLPGTAPKLLIYGNSNRPSGVPDRFSGSKSGTSASLAITGLQAEDEADYYCQSYDSSLSGWVFGGGTKLTVLG

SEQ ID NO: 63 - protein, 112 aa, Artificial Sequence
  light chain variable region of clone 18
QSVLTQPPSVSGAPGQRVTISCTGSSSNIGAGYDVHWYQQLPGTAPKLLIYGNSNRPSGVPDRFSGSKSGTSASLAITGLQDEDEADYYCQSYDSSLSEYVFGTGTKVTVLG

SEQ ID NO: 64 - protein, 112 aa, Artificial Sequence
  light chain variable region of clone 19
QSVLTQPPSVSGAPGQRVTISCTGSSSNFGAGYDVHWYQQLPGTAPKLLIYGNDNRPSGVPDRFSGSKSGTSASLAITGLQDEDEADYYCQSYDSSLSEYVFGTGTQLTDLG

SEQ ID NO: 65 - protein, 111 aa, Artificial Sequence
  light chain variable region of clone 20
QSALIQPRSVSGSPGQSVTISCTGTSSNVGVYNYVSWYQQHPGKAPKLIIYDVTKRPSGVPDRFSGSKSGNTGSLTISGLQAEDEADYYSCSYAGSYTWVFGPGTKVTVLS

SEQ ID NO: 66 - protein, 113 aa, Artificial Sequence
  light chain variable region of clone 21
QTVVTQPPSVSGAPGQRVTISCTGSSSNIGAGYDVHWYQQLPGTAPKLLIYGNSNRPSGVPDRFSGSKSGTSASLAITGLQAEDEADYYCQSYDSSLSGSGVFGGGTKLTVLG

SEQ ID NO: 67 - protein, 112 aa, Artificial Sequence
  light chain variable region of clone 22
SYELTQPPSASGTPGQRVTISCSGSSSNIGAGYDVHWYQQLPGTAPKLLIYGNSNRPSGVPDRFSGSKSGTSASLAITGLQAEDEADYYCQSYDYNLSGYVSGTGTKVTVLG

SEQ ID NO: 68 - protein, 112 aa, Artificial Sequence
  light chain variable region of clone 23
TYELSQPPSVSGAPGQRVTISCTGSSSNIGADYDVHWYQQLPGTAPKLLIYGNNNRPSGVPDRFSGSKSGTSGSLAITGLRSEDEADYYCAAWDDSLSGYVFGTGTKVTVLG

SEQ ID NO: 69 - protein, 112 aa, Artificial Sequence
  light chain variable region of clone 24
QPVLTQPPSVSGAPGQRVTITCTGSGSNIGAGYDVHWYQQLPGTAPKLLIYGNSNRPSGAPDRVSGSKSGTSASLAITGLQAEDEADYYCQSYDSSLRTYVFGTGTKVTVLG

SEQ ID NO: 70 - protein, 112 aa, Artificial Sequence
  light chain variable region of clone 25
QSVLTQPPSVSGAPGQRVTISCTGSSSNIGAGYDVHWYQQLPGTAPKLLIYGNSNRPSGVPDRFSGSKSGTSASLAITGLQAEDEADYYCQSYDSSLSGRVFGGGTKLTVLG

SEQ ID NO: 71 - protein, 112 aa, Artificial Sequence
  light chain variable region of clone 26
QSVLTQPPSVSGAPGQRVTISCTGSSSNIGAGYDVHWYQQLPGTAPKLLIYGNSNRPSGVPDRFSGSKSGTSASLAITGLQAEDEADYYCQSYDSNLSGYVFGTGTKVTVLG

SEQ ID NO: 72 - protein, 112 aa, Artificial Sequence
  light chain variable region of clone 27
SYELMQPPSVSGAPGQRVTISCTGSSSNIGAGYDVHWYQQLPGTAPKLLIYGNSNRPSGVPDRFSGSKSGTSASLAITGLQAEDEADYYCQSYDSSLRAYVFGTGTKVTDLG

SEQ ID NO: 73 - protein, 109 aa, Artificial Sequence
  light chain variable region of clone 28
DVVMTQSPSSLSASVGDRVTITCRASQGITNDLAWYQQKPGKAPKLLIYAASTLQSGVPSRFSGSGSGTDFTLTISSLQPEDFATYYCQQSYDTPPYTFGQGTKLEIKR

SEQ ID NO: 74 - protein, 113 aa, Artificial Sequence
  light chain variable region of clone 29
QSVLTQPPSVSGAPGQRVTISCTGSSSNIGAGYDVHWYQQLPGTAPKLLIYGNSNRPSGVPDRFSGSKSGTSASLAITGLQAEDEADYYCQSYDSSLSGSTVFGGGTELTVLG

SEQ ID NO: 75 - protein, 111 aa, Artificial Sequence
  light chain variable region of clone 30
SYELTQPPSVSGAPGQRVTISCTGSSSNIGAGYDVHWYQQLPGTAPKLLIYGNSNRPSGVPDRFSGSKSGTSASLAITGLQAEDEADYYCQSYDNSLSGVFGGGTKLTVLG

SEQ ID NO: 76 - protein, 113 aa, Artificial Sequence
  light chain variable region of clone 31
QSVLTQPPSVSGAPGQRVTISCTGSSSNIGAGYDVHWYQQVPGTAPKLLIYGNINRPSGVPDRFSGSKSGTSASLAITGLQAEDEADYYCQSYDSSLSGSYVFGTGTKVTVLG

SEQ ID NO: 77 - protein, 112 aa, Artificial Sequence
  light chain variable region of clone 32
QSVLTQPPSVSGAPGQRVTISCTGSSSNIGAGYDVHWYQHLPGTAPKLLIYGNSNRPSGVPDRFSGSKSGTSASLAITGLQAEDEADYYCQSYDGSLSGWVFGGGTKLTVLG

SEQ ID NO: 78 - protein, 108 aa, Artificial Sequence
  light chain variable region of clone 33
AIQLTQSPSSLSASVGDRVTITCRASQSISSYLNWYQQKPGKAPKLLIYAASSLQSGVPSRFSGSGSGTDFTLTISSLQPEDFATYYCQQSYSTPLTFGGGTKVEIKR

SEQ ID NO: 79 - protein, 111 aa, Artificial Sequence
  light chain variable region of clone 34
QPVLTQPPSASGTPGQRVIISCSGSSSNIGSHTVNWYQQLPGTAPKLLIYNNNQRPSGVPDRFSGSKSGTSASLAISGLQSADEADYSCAAWDDSLNGYVFGTGTKVTVLG

SEQ ID NO: 80 - protein, 111 aa, Artificial Sequence
  light chain variable region of clone 35
QSALTQPASVSGSPGQSITISCTGTSSDVGGYNYVSWYQQHPGKAPKLMIYDVGQRPSGVSNRFSGSKSGNTASLTISGLQAEDEADYYCSSYTSSSSYVFGTGTKVTVLG

SEQ ID NO: 81 - protein, 109 aa, Artificial Sequence
  light chain variable region of clone 36
SYELTQPPSVSVAPGKTARITCGGNNIGSKSVHWYQQKPGQAPVLVVYDDSDRPSGIPERFSGSNSGNTATLTISRVEAGDEADYYCQVWDSSSDHVVFGGGTQLIILG

SEQ ID NO: 82 - protein, 111 aa, Artificial Sequence
  light chain variable region of clone 37
RPVLTQPPSASGTPGQRATISCSGSSSNIGSNTVNWYRQLPGTAPKLLIHSNNQRPSGVPDRFSGSKSGTSASLAISGLQSEDEADYYCATWDDSLDGWVFGGGTKLTVLG

SEQ ID NO: 83 - protein, 111 aa, Artificial Sequence
  light chain variable region of clone 38
QTVVTQEPSVSAAPEQKVTISCSGSSSNIGNNYVSWYQQLPGTAPKLLIYDNNKRPSGIPDRFSGSKSGTSATLGITGLQTGDEADYYCGTWDSSLSAYVFGTGTKVTVLG

SEQ ID NO: 84 - protein, 111 aa, Artificial Sequence
  light chain variable region of clone 39
QSVLTQPPSVSAAPGQKVTISCSGSGSNVENNYVSWYQQLPGTAPKLLIYENNNRPSGIPDRFSGSKSGTSATLGITGLQTGDEADYYCGVWDDSLNHVIFGGGTKLTVLG

SEQ ID NO: 85 - protein, 108 aa, Artificial Sequence
  light chain variable region of clone 40
EIVLTQSPSSLSASVGDRVTITCRASQSISSYLNWYQQKPGKAPKLLIYAASSLQSGVPSRFSGSGSGTDFTLTISSLQPEDFATYYCQQSYSTPRTFGQGTRLEIKR

SEQ ID NO: 86 - protein, 107 aa, Artificial Sequence
  light chain variable region of clone 41
SYELTQPPSVSVAPGKTARITCGGNNIGSKSVHWYQQKPGQAPVLVVYDDSDRPSGIPERFSGSNSGNTATLTISRVEAGDEADYYCQVWDSSSVVFGGGTKLTVLG

SEQ ID NO: 87 - protein, 121 aa, Artificial Sequence
  heavy chain variable region of clone M1
EVQLVESGGGLVQPGGSLRLSCAASGFTFSTYYMGWVRQAPGKGLEWVSLISGSGGSTYYDDSVKGRFTISRDNSKNTLYLQMNSLRAEDTAVYYCAKPPYSFDSMSESDYWGQGTLVTVS

SEQ ID NO: 88 - protein, 115 aa, Artificial Sequence
  heavy chain variable region of clone M2
QAYLQQSGAELVRSGASVKLSCTASGFNIKDYYMHWVKQRPEQGLEWIGWIDPENGDTEYAPKFQGKATMTADTSSNTAYLQLSSLTSEDTAVYYCNEDGNYDYWGQGTTLTVSS

SEQ ID NO: 89 - protein, 111 aa, Artificial Sequence
  heavy chain variable region of clone M3
EVQLLESGGGLVKPGGSLKLSCAASGFTFSSYDMSWVRQTPEKRLDWVASISSSGGTYYPDSVKGRFTISRDIARNILYLQMNSLRSEDTAMYYCVRGDYWGQGTTLTVSS

SEQ ID NO: 90 - protein, 117 aa, Artificial Sequence
  heavy chain variable region of clone M4
DVMLVESGGDLVKPGGSLKLSCAASGFTFSSRGMSWVRQTPDKRLEWVATISFGDIYTYYPDSVKGRFTISRDNAKNTLYLQMSSLKSEDTAIYYCVRPNDGYFDYWGQGTTLTVSA

SEQ ID NO: 91 - protein, 117 aa, Artificial Sequence
  heavy chain variable region of clone M5
EVKLVESGGDLVKPGGSLKLSCAASGFTFSSRGMSWVRQTPDKRLEWVATISFGDIYTYYPDSVKGRFTISRDNAKNTLYLQMSSLKSEDTAIYYCARPNDGYFDYWGQGTTLTVSS

SEQ ID NO: 92 - protein, 111 aa, Artificial Sequence; identical to SEQ ID NO: 84
  light chain variable region of clone M1

SEQ ID NO: 93 - protein, 112 aa, Artificial Sequence
  light chain variable region of clone M2
DVVVTQSPASLAVSLGQRATISCKASQSVDYAGDSYMNWYQQKPGQPPKLLIYAASNLESGIPARFSGSGSGTDFTLNIHPVEEEDAATYYCQQSNEDPWTFGGGTKLEIKR

SEQ ID NO: 94 - protein, 108 aa, Artificial Sequence
  light chain variable region of clone M3
DIVMTQSHKFMSASVGDRVNITCKASQDVGTAVAWYQQKPGQSPKLLIYWASTRHTGVPDRFTGSGSGTDFTLTISNVQSEDLADYFCQQYTRYSNTFGGGTKLEIKR

SEQ ID NO: 95 - protein, 108 aa, Artificial Sequence
  light chain variable region of clone M4
DIVMTQSHKFMSTSVGDRVSITCKASQDVSTDVAWYQQKPGQSPKLLIYWASTRHTGVPDRFTGSGSGTDYTLTINSVQAEDLALYYCQQHYSTPWTFGGGTKLEIKR

SEQ ID NO: 96 - protein, 107 aa, Artificial Sequence
  light chain variable region of clone M5
DVVMTQTPKFLLVSAGDRVTITCKASQSVSNDVAWYQQKPGQSPKLLIYYASNRYTGVPDRFTGSGYGTDFTLTINSVQAEDLAVYYCQQSYSAPYTFGGGTKLEMK

SEQ ID NO: 97 - protein, 119 aa, Artificial Sequence
  heavy chain variable region of clone 5E9
EVQLVESGGGLVQPGGSLRLSCAASGFTFTTYDMGWVRQAPGKGPEWVSLISSGGSNTWYDDSVKGRFTISRDNSKNTLYLQMNSLRAEDTAVYYCAKEKYPYSDCDYWGQGTLVTVSS

SEQ ID NO: 98 - protein, 117 aa, Artificial Sequence
  heavy chain variable region of clone 6D9
EVQLVESGGGLVQPGGSLRLSCAASGFTFTDYDMGWVRQAPGKGPEWVSLISGDSGNTWYDDSVKGRFTISRDNSKNTLYLQMNSLRAEDTAVYYCAKYRGTTKDYWGQGTLVTVSS

SEQ ID NO: 99 - protein, 112 aa, Artificial Sequence
  heavy chain variable region of clone 6H10
EVQLVESGGGLVQPGGSLRLSCAASGFTFTNYYMGWVRQAPGKGPEWVSLISYDGSSTWYDDSVKGRFAISRDNSKNTLYLQMNTLRAEDTAVYYCAKPDYWGQGTLVTVSS

SEQ ID NO: 100 - protein, 117 aa, Artificial Sequence; identical to SEQ ID NO: 90
  heavy chain variable region of clone M4-1 (H original)

SEQ ID NO: 101 - protein, 117 aa, Artificial Sequence; identical to SEQ ID NO: 90
  heavy chain variable region of clone M4-2 (H original)

SEQ ID NO: 102 - protein, 117 aa, Artificial Sequence
  heavy chain variable region of clone M4-3 (H1)
EVQLVESGGGLVKPGGSLRLSCAASGFTFSSRGMSWVRQAPGKGLEWVSTISFGDIYTYYPDSVKGRFTISRDNAKNSLYLQMNSLRAEDTAVYYCARPNDGYFDYWGQGTLVTVSS

SEQ ID NO: 103 - protein, 117 aa, Artificial Sequence; identical to SEQ ID NO: 102
  heavy chain variable region of clone M4-4 (H1)

SEQ ID NO: 104 - protein, 117 aa, Artificial Sequence; identical to SEQ ID NO: 102
  heavy chain variable region of clone M4-5 (H1)

SEQ ID NO: 105 - protein, 117 aa, Artificial Sequence
  heavy chain variable region of clone M4-6 (H2)
EVQLVESGGGLVKPGGSLKLSCAASGFTFSSRGMSWVRQAPGKGLEWVATISFGDIYTYYPDSVKGRFTISRDNAKNSLYLQMNSLKAEDTAIYYCARPNDGYFDYWGQGTLVTVSS

SEQ ID NO: 106 - protein, 117 aa, Artificial Sequence; identical to SEQ ID NO: 105
  heavy chain variable region of clone M4-7 (H2)

SEQ ID NO: 107 - protein, 117 aa, Artificial Sequence; identical to SEQ ID NO: 105
  heavy chain variable region of clone M4-8 (H2)

SEQ ID NO: 108 - protein, 117 aa, Artificial Sequence; identical to SEQ ID NO: 91
  heavy chain variable region of clone M5-1 (H original)

SEQ ID NO: 109 - protein, 117 aa, Artificial Sequence; identical to SEQ ID NO: 91
  heavy chain variable region of clone M5-2 (H original)

SEQ ID NO: 110 - protein, 117 aa, Artificial Sequence; identical to SEQ ID NO: 102
  heavy chain variable region of clone M5-3 (H1)

SEQ ID NO: 111 - protein, 117 aa, Artificial Sequence; identical to SEQ ID NO: 102
  heavy chain variable region of clone M5-4 (H1)

SEQ ID NO: 112 - protein, 117 aa, Artificial Sequence; identical to SEQ ID NO: 102
  heavy chain variable region of clone M5-5 (H1)

SEQ ID NO: 113 - protein, 117 aa, Artificial Sequence; identical to SEQ ID NO: 105
  heavy chain variable region of clone M5-6 (H2)

SEQ ID NO: 114 - protein, 117 aa, Artificial Sequence; identical to SEQ ID NO: 105
  heavy chain variable region of clone M5-7 (H2)

SEQ ID NO: 115 - protein, 117 aa, Artificial Sequence; identical to SEQ ID NO: 105
  heavy chain variable region of clone M5-8 (H2)

SEQ ID NO: 116 - protein, 108 aa, Artificial Sequence
  light chain variable region of clone M4-1 (hM4-k2)
DIVMTQSPATLSVSPGERATLSCKASQDVSTDVAWYQQKPGQAPRLLIYWASTRHTGVPDRFSGSGSGTDFTLTISSLQSEDFAVYYCQQHYSTPWTFGGGTKVEIKR

SEQ ID NO: 117 - protein, 108 aa, Artificial Sequence
  light chain variable region of clone M4-2 (hM4-k3)
DIVMTQSPATLSVSPGDRVSISCRASQDVSTDVAWYQQKPGQSPKLLIYWASTRHTGVPDRFTGSGSGTDYTLTISSLQPEDFAVYYCQQHYSTPWTFGGGTKVEIKR

SEQ ID NO: 118 - protein, 108 aa, Artificial Sequence; identical to SEQ ID NO: 95
  light chain variable region of clone M4-3 (4k original)

SEQ ID NO: 119 - protein, 108 aa, Artificial Sequence; identical to SEQ ID NO: 116
  light chain variable region of clone M4-4 (hM4-k2)

SEQ ID NO: 120 - protein, 108 aa, Artificial Sequence; identical to SEQ ID NO: 117
  light chain variable region of clone M4-5 (hM4-k3)

SEQ ID NO: 121 - protein, 108 aa, Artificial Sequence; identical to SEQ ID NO: 95
  light chain variable region of clone M4-6 (4k original)

SEQ ID NO: 122 - protein, 108 aa, Artificial Sequence; identical to SEQ ID NO: 116
  light chain variable region of clone M4-7 (hM4-k2)

SEQ ID NO: 123 - protein, 108 aa, Artificial Sequence; identical to SEQ ID NO: 117
  light chain variable region of clone M4-8 (hM4-k3)

SEQ ID NO: 124 - protein, 108 aa, Artificial Sequence
  light chain variable region of clone M5-1 (hM5-k1)
DIQMTQSPSSLSASVGDRVTITCKASQSVSNDVAWYQQKPGKAPKLLIYYASNRYTGVPSRFSGSGSGTDFTLTISSLQPEDFATYYCQQSYSAPYTFGGGTKVEIKR

SEQ ID NO: 125 - protein, 108 aa, Artificial Sequence
  light chain variable region of clone M5-2 (hM5-k2)
DVVMTQSPATLSVSPGERATLSCKASQSVSNDVAWYQQKPGQAPRLLIYYASNRYTGVPDRFTGSGSGTDFTLTISSLQSEDFAVYYCQQSYSAPYTFGGGTKVEIKR

SEQ ID NO: 126 - protein, 107 aa, Artificial Sequence; identical to SEQ ID NO: 96
  light chain variable region of clone M5-3 (5k original)

SEQ ID NO: 127 - protein, 108 aa, Artificial Sequence; identical to SEQ ID NO: 124
  light chain variable region of clone M5-4 (hM5-k1)

SEQ ID NO: 128 - protein, 108 aa, Artificial Sequence; identical to SEQ ID NO: 125
  light chain variable region of clone M5-5 (hM5-k2)

SEQ ID NO: 129 - protein, 107 aa, Artificial Sequence; identical to SEQ ID NO: 96
  light chain variable region of clone M5-6 (5k original)

SEQ ID NO: 130 - protein, 108 aa, Artificial Sequence; identical to SEQ ID NO: 124
  light chain variable region of clone M5-7 (hM5-k1)

SEQ ID NO: 131 - protein, 108 aa, Artificial Sequence; identical to SEQ ID NO: 125
  light chain variable region of clone M5-8 (hM5-k2)

SEQ ID NO: 132 - DNA, 408 bp, Artificial Sequence
  H1
tgctgtgggtgagtggtacctgtggggaagtccaactggttgagtccggtggaggactcgtcaagcccggtgggtctctccgactgagttgtgcggcatctggcttcactttctccagtcgaggtatgtcttgggttcgacaagcgccagggaaagggctggaatgggtcagtaccatatctttcggggacatatatacctattacccggattctgtgaaaggaaggtttactataagtcgggataatgcaaagaactccttgtatcttcaaatgaactccctgcgagctgaggatactgcagtctactattgtgcccggcccaatgacgggtattttgactactggggccaaggtactctggttacggttagttcagcctccaccaagggcccatcggtcttccccc

SEQ ID NO: 133 - DNA, 408 bp, Artificial Sequence
  H2
tgctgtgggtgagtggtacctgtggggaagtccaactggttgagtccggtggaggactcgtcaagcccggtgggtctctcaaactgagttgtgcggcatctggcttcactttctccagtcgaggtatgtcttgggttcgacaagcgccagggaaagggctggaatgggtcagtaccatatctttcggggacatatatacctattacccggattctgtgaaaggaaggtttactataagtcgggataatgcaaagaactccttgtatcttcaaatgaactccctgaaagctgaggatactgcagtctactattgtgcccggcccaatgacgggtattttgactactggggccaaggtactctggttacggttagttcagcctccaccaagggcccatcggtcttccccc

SEQ ID NO: 134 - DNA, 370 bp, Artificial Sequence
  hM4-k1
tgctgtgggtgagtggtacctgtggggatatacagatgacccagtctccgtctagtctgagcgcgtccgtgggcgatcgggttactattacttgcaaggccagccaggatgtatctacagacgtagcctggtatcagcaaaaaccaggcaaagctcccaaactgcttatatattgggcgagtacccgacatacgggggtcccgagcaggtttagtggttctgggtccgggacagactttactttgaccattagttccctgcagcccgaggactttgccacttattactgtcagcagcactatagcacgccttggactttcgggggaggtacaaaagttgaaatcaagcgtacggtggccgctccaagcgt

SEQ ID NO: 135 - DNA, 370 bp, Artificial Sequence
  hM4-k2
tgctgtgggtgagtggtacctgtggggatatagtgatgactcaaagcccggcgacgctttccgtttctcccggtgagcgggcaaccttgtcatgcaaagcatcccaggatgtttccacggacgtggcatggtatcaacaaaagccaggtcaagcgccacgcctccttatatactgggcatcaactcgacacaccggggtgccggacaggttcagcggaagcgggagcggtacagacttcactctcaccattagttcattgcagagcgaggactttgctgtttactactgccaacaacactatagcacgccctggacattcgggggcggaacgaaagtggagatcaagcgtacggtggccgctccaagcgt

SEQ ID NO: 136 - DNA, 370 bp, Artificial Sequence
  hM4-k3
tgctgtgggtgagtggtacctgtggggatatagtgatgactcaaagcccggcgacgctttccgtttctcccggtgaccgggtaagcttgtcatgcagagcatcccaggatgtttccacggacgtggcatggtatcaacaaaagccaggtcaaagcccacgcctccttatatactgggcatcaactcgacacaccggggtgccggacaggttcagcggaagcgggagcggtacagacttcactctcaccattagttcattgcagcccgaggactttgctgtttactactgccaacaacactatagcacgccctggacattcgggggcggaacgaaagtggagatcaagcgtacggtggccgctccaagcgt

SEQ ID NO: 137 - DNA, 370 bp, Artificial Sequence
  hM5-k1
tgctgtgggtgagtggtacctgtggggacatacagatgacgcagtcaccgtcttcactctccgccagcgtaggtgaccgggtcactattacctgtaaagcctcccaaagcgtttcaaatgacgtcgcctggtatcagcagaaaccgggaaaagcgcccaaattgcttatatactacgccagtaaccgatataccggtgttccatcacgctttagcgggagcggcagtggtactgactttacattgacaattagttcccttcaacctgaggattttgcaacttattactgccagcagagttattctgccccctatacattcggtggggggacgaaggtggagataaagcgtacggtggccgctccaagcgt

SEQ ID NO: 138 - DNA, 370 bp, Artificial Sequence
  hM5-k2
tgctgtgggtgagtggtacctgtggggacgttgtaatgacgcaatctcccgctaccttgtccgtctcaccaggtgagagggcaaccctgagttgtaaagcaagtcagtccgtgtcaaacgatgtcgcctggtatcaacagaagcccggccaagctccccgattgcttatctactacgcaagtaaccgctatacaggcgtcccggatcggttcacggggagtggcagtggcacggatttcaccctgacaatatcttctctccaaagtgaggactttgcggtgtactactgtcagcagtcatactctgccccatatacttttggcggtgggactaaggttgaaattaaacgtacggtggccgctccaagcgt

SEQ ID NO: 139 - protein, 5 aa, Artificial Sequence
  VH-CDR1 of M4, M5, and M4-4
SRGMS

SEQ ID NO: 140 - protein, 17 aa, Artificial Sequence
  VH-CDR2 of M4, M5, and M4-4
TISFGDIYTYYPDSVKG

SEQ ID NO: 141 - protein, 8 aa, Artificial Sequence
  VH-CDR3 of M4, M5, and M4-4
PNDGYFDY

SEQ ID NO: 142 - protein, 11 aa, Artificial Sequence
  VL-CDR1 of M4, and M4-4
KASQDVSTDVA

SEQ ID NO: 143 - protein, 7 aa, Artificial Sequence
  VL-CDR2 of M4, and M4-4
WASTRHT

SEQ ID NO: 144 - protein, 9 aa, Artificial Sequence
  VL-CDR3 of M4, and M4-4
QQHYSTPWT

SEQ ID NO: 145 - protein, 11 aa, Artificial Sequence
  VL-CDR1 of M5
KASQSVSNDVA

SEQ ID NO: 146 - protein, 7 aa, Artificial Sequence
  VL-CDR2 of M5
YASNRYT

SEQ ID NO: 147 - protein, 9 aa, Artificial Sequence
  VL-CDR3 of M5
QQSYSAPYT

SEQ ID NO: 148 - protein, 30 aa, Artificial Sequence
  VH-FR1 of M4
DVMLVESGGDLVKPGGSLKLSCAASGFTFS

SEQ ID NO: 149 - protein, 14 aa, Artificial Sequence
  VH-FR2 of M4, and M5
WVRQTPDKRLEWVA

SEQ ID NO: 150 - protein, 32 aa, Artificial Sequence
  VH-FR3 of M4
RFTISRDNAKNTLYLQMSSLKSEDTAIYYCVR

SEQ ID NO: 151 - protein, 11 aa, Artificial Sequence
  VH-FR4 of M4
WGQGTTLTVSA

SEQ ID NO: 152 - protein, 30 aa, Artificial Sequence
  VH-FR1 of M5
EVKLVESGGDLVKPGGSLKLSCAASGFTFS

SEQ ID NO: 153 - protein, 32 aa, Artificial Sequence
  VH-FR3 of M5
RFTISRDNAKNTLYLQMSSLKSEDTAIYYCAR

SEQ ID NO: 154 - protein, 11 aa, Artificial Sequence
  VH-FR4 of M5
WGQGTTLTVSS

SEQ ID NO: 155 - protein, 30 aa, Artificial Sequence
  VH-FR1 of M4-4
EVQLVESGGGLVKPGGSLRLSCAASGFTFS

SEQ ID NO: 156 - protein, 14 aa, Artificial Sequence
  VH-FR2 of M4-4
WVRQAPGKGLEWVS

SEQ ID NO: 157 - protein, 32 aa, Artificial Sequence
  VH-FR3 of M4-4
RFTISRDNAKNSLYLQMNSLRAEDTAVYYCAR

SEQ ID NO: 158 - protein, 11 aa, Artificial Sequence
  VH-FR4 of M4-4
WGQGTLVTVSS

SEQ ID NO: 159 - protein, 23 aa, Artificial Sequence
  VL-FR1 of M4
DIVMTQSHKFMSTSVGDRVSITC

SEQ ID NO: 160 - protein, 15 aa, Artificial Sequence
  VL-FR2 of M4, and M5
WYQQKPGQSPKLLIY

SEQ ID NO: 161 - protein, 32 aa, Artificial Sequence
  VL-FR3 of M4
GVPDRFTGSGSGTDYTLTINSVQAEDLALYYC

SEQ ID NO: 162 - protein, 11 aa, Artificial Sequence
  VL-FR4 of M4
FGGGTKLEIKR

SEQ ID NO: 163 - protein, 23 aa, Artificial Sequence
  VL-FR1 of M5
DVVMTQTPKFLLVSAGDRVTITC

SEQ ID NO: 164 - protein, 32 aa, Artificial Sequence
  VL-FR3 of M5
GVPDRFTGSGYGTDFTLTINSVQAEDLAVYYC

SEQ ID NO: 165 - protein, 10 aa, Artificial Sequence
  VL-FR4 of M5
FGGGTKLEMK

SEQ ID NO: 166 - protein, 23 aa, Artificial Sequence
  VL-FR1 of M4-4
DIVMTQSPATLSVSPGERATLSC

SEQ ID NO: 167 - protein, 15 aa, Artificial Sequence
  VL-FR2 of M4-4
WYQQKPGQAPRLLIY

SEQ ID NO: 168 - protein, 32 aa, Artificial Sequence
  VL-FR3 of M4-4
GVPDRFSGSGSGTDFTLTISSLQSEDFAVYYC

SEQ ID NO: 169 - protein, 11 aa, Artificial Sequence
  VL-FR4 of M4-4
FGGGTKVEIKR